European Patent Specification EP 3 523 428 B1, published January 10, 2024. Title: TOBACCO PLANTS HAVING INCREASED NITROGEN EFFICIENCY AND METHODS OF USING SUCH PLANTS. Applicant: Altria Client Services LLC. The sequence listing filed with the application follows.

SEQUENCE LISTING (20 sequences)

SEQ ID NO: 1 - DNA, 738 bp, Nicotiana tabacum
atgccttcagacgtaagtgaacgaaaagctaccaaacaacagcaaggagctgcaccggcaccggagccggagcatcttccatgtccacgctgtgattccaccaacactaaattctgctactacaacaactacaacttctctcagccacgtcacttctgtaagtcctgccgccgttattggacacacggcggcactcttcgtgacatccccgttggtgggggtagtcgcaaaaatgccaaacgctcccgtacaatcactactaacaacaccagtagcagcactagcagctgcttgtcctccacgctctctcctcgcgactaccatcacgcgcctactccatcacacgtttctccatttttggttcctctaactgccgatcatcacggcgggccactaccctttgacgtgaagccgaatgggaacatgtgtgggagtttcacctcgttgttgagcaatactcaagggcctcatggtcttttagcactcagtgggttcgggcttggagttgggcctgcaattgaagatatgggctttggtcttggaaggcccatatggccatttcctggagtagtgtcgcataccagtgttgatcatagtaacagtaacggtgctggagctagtatgttgggcaacacgtggcagcttgctagtggagaaggtggatttgttggagctggaggagattgttttaatttcccagaacttgctatttcaacgcatggaaatggtatgaaatga

SEQ ID NO: 2 - DNA, 738 bp, Nicotiana tabacum; identical to SEQ ID NO: 1

SEQ ID NO: 3 - protein, 245 aa, Nicotiana tabacum
MPSDVSERKATKQQQGAAPAPEPEHLPCPRCDSTNTKFCYYNNYNFSQPRHFCKSCRRYWTHGGTLRDIPVGGGSRKNAKRSRTITTNNTSSSTSSCLSSTLSPRDYHHAPTPSHVSPFLVPLTADHHGGPLPFDVKPNGNMCGSFTSLLSNTQGPHGLLALSGFGLGVGPAIEDMGFGLGRPIWPFPGVVSHTSVDHSNSNGAGASMLGNTWQLASGEGGFVGAGGDCFNFPELAISTHGNGMK

SEQ ID NO: 4 - DNA, 804 bp, Artificial Sequence
  synthetically-generated oligonucleotide
acggatccacaagcgagaagaaaaatgccttcagacgtaagtgaacgaaaagctaccaaacaacagcaaggagctgcaccggcaccggagccggagcatcttccatgtccacgctgtgattccaccaacactaaattctgctactacaacaactacaacttctctcagccacgtcacttctgtaagtcctgccgccgttattggacacacggcggcactcttcgtgacatccccgttggtgggggtagtcgcaaaaatgccaaacgctcccgtacaatcactactaacaacaccagtagcagcactagcactgcttgtcctccacgctctctcctcgcgactaccatcacgcgcctactccatcacacgtttctccatttttggttcctctaactgccgatcatcacggcgggccactaccctttgacgtgaagccgaatgggaacatgtgtgggagtttcacctcgttgttgagcaatactcaagggcctcatggtcttttagcactcagtgggttcgggcttggagttgggcctgcaattgaagatatgggctttggtcttggaaggcccatatggccatttcctggagtagtgtcgcataccagtgttgatcatagtacagtaacggtgctggagctagtatgttgggcaacacgtggcagcttgctagtggagaaggtggatttgttggagctggaggagattgttttaatttcccagaacttgctatttcaacgcatggaaatggtatgaaatgattgtttaaggatggtatgaaatgattgtttaaggattctagagt

SEQ ID NO: 5 - DNA, 903 bp, Nicotiana tabacum
atgttttctgggttctcccatttcagttgtgatgcaatcaacgcctgttgggccgctcctgtcctaatatcgttaaatattgcactgaagtgtgtaaaaaagcaatctttatctactgaagctattgaagagcggttagctggagtacctgtttatgcacttagcaatgcttctgaagaattcgtgcttgtttcgggtgttagtactggtaaaaatcttgggttattttgctttagtgaagctgatgctgaagctcttcgtcagcaaatggaatctatggaccctactatgcgaaatggctcgagggttgttcctgttgctcttaataaggttttccagctcaaagttgatggagtggcttttaggctgataccagaggcatctcaagtaaagaatgcaatgaaggaaagggaaaggactggaacgtctgatgagagcttttatggtgttccagtgtttcagtcaaggagcttaattctgaggagccagaacaagagatatcgccctgttttcttcaggaaggaggacctagagaattcactagtaagagcttctcaacagcaaggccgattgaatcctgctttgaaaggagatattcaggttgctgttctggaggatataatacaaggcatgaaggatacttcgacgtcaaagtgggacgatgttgtatttgttcctccgggtttcgatgtttcaacagatccttcccagaataactttgactatgcattaggtcctgttatgcgacaaattcttatagaaaccggagctaagatttctgaagtgtttgataattgtagacaaattctgtgtgcaattaacttctctcactcgaagtgtgacgttaatctcgatagcagtggtgatgtgtatgttattgataagctttacattttgagctga

SEQ ID NO: 6 - DNA, 8144 bp, Nicotiana tabacum
atgttttctgggttctcccatttcagttgtgatgcaatcaacgttaaattcatttaattttttgtactttataaaactaagttctcattttttttaatttcacatcctcacttgtctaatttttaaaaaaataatattcattaaatataatatatatatatatatattaaggcctcttattaagtgtttgttttaggcctgttgggccgctcctgtcctaatatcgttaaatattgcactgaagtggtaagttactcatgcatctttaattaaatattttgaattagaattaaaagaataaaattacctttgataataagcactttaccccaatagattttttaagccgtatgggtaaataaaacactcttaatataggtaaacaatttcctttttaccttgcctctctctctatcttttgttcccacccacccccacaccctcaccccctaccccccaccctctccccttttcttctagacgcaaaatctttagcagtttttaaaacctccaaaacccttttcaccattttctctctaatttcaactaaaacagaggagaaaaaaaaacatgaatatcttcaaacctaaacagtcatcttcttcttcagcaacaccacgtcaccaccacatctacagctccaacaaactttcaagaatttacaaacccatttctccaatttccttcaaaccacttttccgcaactcaacacactcaattcttctcaaaattcacaaaacccatgggctaaaattggtgttaataataataatagtgtaaaaaagcaatctttatctactgaagctattgaagagcggttagctggagtacctgtttatgcacttagcaatgcttctgaagaattcgtgcttgtttcgggtgttagtactggtaaaaatcttgggttattttgctttagtgaagctgatgctgaagctcttcgtcagcaaatggaatctatggaccctactatgcgaaatggctcgagggttgttcctgttgctcttaataaggttagcttcattaattgcttttctacaaccccattttttgtgtaatggatgtgcttattgtgttatgattaacagtagtgaagccagaaaattcaataagagtgttcaaattttgaacaacctttgtcagtgggctatgcaaggtgttcaaagtcttttttattaataacaagtaatatttgaccctatatacagaataattttaaagggtgttcagttgaccactcttggccacacatagcttcatccgtgatgattaactatgctcgacaagtagtgttatgtcgggtcaatgaagtgggatgagaaccatagcggaggcaaaagaacactaggtaatttttccttagtggatagagttatcttgtacctttgctggtgggagctagtagatacatgtagaataggtgcgcgcaagttggcacagacaccactgtcattagaaaaacttaagaaaattaaaaaatagtgttcggggggttagtacacgactacacggacttgttgtgtgtcgaatataataaatgaattgtttatgtgaggaataataatgcgaggattgttatagggtgaaaaagaatatagagattgttatgggttgagtactattgcagggatttttatgcatagattgcctacttaatatttgttcccgttgctctcgataaggttaaatttattggctgcgattggccccgacatcacagtcatctgaaaaagaaaagtaataacaaatagtgtcaaatagtgttagcggggttagcacatggactaattttgctgcgattataatgaaggatttgtttatgtggagaacaaagacaaaaatgtagggattgttatgcattgagtactagtgtggggattattatgcgtagattgcctacgtataggaatttttgtctttagatatttttatctatgtattctaatacacgtttcctattctacattctattttgcacgaaataatatatagattcctgcaaagcttacaagggtactggcaatgtggagtttaaactgccaatcaaatgctacattaatatacaaagattgtttttccttaggcagctaaacaaacattgaatttactttgtggaatttcatgttgagattatatttttatgcggcaataacgtgagcccttataaaacgtgtgtttgacttaacatgattattaagagaaacaagaattatgtcttaatcctaagttgtgattgactatataaatccccaataatcatttcgttccatttggcccgtcccatttcaattcaatgatttgggtttctctaaaccggaggttctttacattctttaagtgaaatataaatttttaaacaaactaaaaagacttgtaacaaacactaaactggtctgtagtgtactgacatgattatctcttaatcgaaaatatgggtgttttgggaatcaaagagcttaaaatttagagtaagaactgagaataagaattgtttaacatttgctgagaaatagccatgtgtttactttttataactagaacaatgacgtaaagataatatggtattggaaagaacaaaagcaagtaggacaagcatgtctaagctagtaattgtcgttgttgaatttaaatactgattatcagaggctgatagttgtattctttattgcgaaagaaaaatgttattaagtctaattgatggtcaataatgcaggttttccagctcaaagttgatggagtggcttttaggctgataccagaggcatctcaagtaaagaatgcaatgaaggtgaatatctgatgataaagatttctgtaatttttattcatgaagtcaatgttttgattttggtttgaaattctctggctgcagactaagtgtgtgcttaaatctttaagaaagctgataaagtactcatgtactcatgtcatcatgttagtatcgtgagaatttgaaattcggttgcttgtcgatcttcaagaagtgctgtctataggtcaatcagtttcttatgttcttaatcaaaaaagggcagcccggtgcactaagctcccgctatgcacccgaaaaaggccggaccacaagggtttattatacgcaacctttatcttcatttctgtaagaggctgtttccacggctcgaacccgtgacctcctggtcacatgacaacaactttactagttacaccaaggctccccttcgttcttaatcaaacaaaagattattcattttggaggtctccattagtctattatagtagagtatcatagctttccaggatcaggtattacctattctctgcttgctgagcatagtcatgatcattgcaaagtatttgcaggtattccaaagttttcgacaatctaagttctgaaatgtacttcatggccattggtcaagattttgaaagttttagtatcattatctatgaaacttttacacaatttgtatgttttaattagcatattacacactcttttattgttctagctctcccttttatgcaaccaatgtgcgagcattggttgcatacactgtcaagcataagattcttccagtttcagtacttcgtactgtcgatgattttaacatcctgtcctttgcggagtggttttcttgttcttactagtagcattagtacgccttgtcgtattgttttcagtcttaggtttctattattgtctgttgttgctttcattttggtcatcttactatcttctgttatcaatgcttcttttccatggctcctcactattgtttctggctgttttcatttcattactgttgagcttattcttcactgagccgagggtctatgggaaacaaaatctctatctccacgcttcttttccatggctcctcactattgtttctagctgttttcatttcattactgttgagcttattcttcactgagccgagggtctatgggaaacaaaatctctatctccacgagatagggtaaggtctgcgtacacactgccctccccagaccccactatgtgggattacactatgttttttgttgttgttgctgctgctgtgtgagcacttttggttattccaagattccttctctataaatatgttatgattgatgattcaacaggaatcctatctaaaacattgtaagaccccgtcttttgtttgactaaatgctaaaaacatccagagtaatgagatagcacaacaataagtagtagatacttttgcttgacgccaaatctgaaaatttgtggcacttcagattagcattaagatgtttttcttcatcttagagataaatatatagtaaacagaagttgcttttgagttgaagtggatgaaaagatagctgttgctcagtaagtttctttttacatgtaccagttgtggactccagaacatagtgtcataacatatattcggtcagtcaaatgttaggaggcctcatctttaagtgatatttctttgaggataacatttaggtttctgcttatgccaaaaatatttttgtgtatccaaatttagttcagcatgtttaaattatcattttgggcgccataactttttcctgctataatctgaagctgatcatattctgctgccattttttttaactaggaaagggaaaggactggaacgtctgatgagagcttttatggtgttccagtgtttcaggtacactctctcagctataatcttggcatcctttagcagctagacaactgccaaagcatgatataaaaagtcggtttagaaactgaaatgctcatctgccttgtcatttgtgcttactgctacgtccccgtgtgtgagtggaaacaaatgcttttttttaccttatcaaaaaaaatctttgaatgacatatgagctcaactaggatccagtaccttcaagaccggaaaagatccaatctgccttaaactgcaattaagagaatccctgtgtgcactaataaatgcccgaaatgattaaaggcaaaaagacatccgcgcaaaatattgcgaagcttcgacctctgcatctgagacagcattgcattgctctcgtttcaccttcttggatgatgttgcctggttaagaaagttcttttgtcgcttgtgtagcagcctgatgcaaatttaactttagaatcatcattaataatgtgaccactactgaggttttaagctagatatcctcttcattcatataagaaagagttctaatggcaaacctatttagtatttccttataggactcgcatgtttgtgccaatatgtttcttattttattcctaaagataccaatctcttattatgaaataagccgatctcttggatgaataagtgcgtaacatttccatgattgaatatgttgaaggatgcaaaaccatctccacaaaccgacatatgggagagttccgatgtttcacagtttgcttaaattttattattcaaaaagaatatcgtggcagacaggattcggatcctagcaaaagcaaaaaagttaggtgatttctttccatttatctaaattttggtaggcagagttatccaattcctatacttgtgagagaatgcaggtatccagtagaatatttgaggtaattttcttataaccgtgggtttaggccaacttgtgcgcaccttgactaattccacggggtacctgctatctccgggggccaccagcacaggtacggggtaactctgtctaccaaggctcgggataaacaccatgcggcagacatctgaaaatcacagtcaaataatttcacaacagatttcgtaccgttaagattcatagattgtgtgaatggtgggctgggaatttcatgccacatgacagccttttttgctatatagccacaaatatagcatactagatcttgtttttcttgtcagttctccttctcatgagtttgaaaattatagtcaaggagcttaattctgaggagccagaacaagagatatcgccctgttttcttcaggaaggttagctaactgtctggagttagtatccactaatgtgatatgatgctatatcgcccttcgtgtaaatttatcaacttgtgcaggaggacctagagaattcactagtaagagcttctcaacagcaaggccgattgaatcctgctttgaaaggagatattcaggtacgtctattgatatttacttaccgttgtgtcttagcttcaagaattatgaccgagaattttcatctgatttcacaggttgctgttctggaggatataatacaaggcatgaaggtgagaatcctcaacaagaaatttacatgttatatcgtcgagttcttgatccaacaaatgatgtcgggaaattatgcagaacttctctgtcgtcctcttactcgttttagtttcttatatatatatatttttgctaatcaagaaattgccaaagccagatagcacatggttcgaaactcagtggataatagccgcccctctacccttttccatttaaataccaagcttttgtatgcaacattgtttgaactcgtgacatgtgcctaactcacacatcatgcgttacgctgttatttatgttcatcttgcttgttaaatgcacattgccttggttaatggccgtaatggagtcggtgcgattaacaaagaatgaacatatttttgcaggatacttcgacgtcaaagtgggacgatgttgtatttgttcctccgggtttcgatgtttcaacagatccttcccagaagtaagagaacctatgtcaagtcatctcatggtgcttggccaatcctatattagcatttttgatatcatgtgtgtaaattgtagtaactttgactatgcattaggtcctgttatgcgacaaattcttatagaaaccggagctaagatttctgaagtgtttgataattgtagacaaattctgtgtgcaattaacttctctgtaggatgtcaaacggtgtggtgcggttgcagggcaaacccgcaaagatttcgccccgcaccgcatcacataatttgttgttttcaacccaccctacctgccccgcataaacccgccccccgtttaagtttttttttttcttttttttcttttttgatagtaaaaactaagattcataaacttctttttcattttttctgaaatagtattaatttaatgtaaacccaaatcctatacaagcacctccctaacaaaaccaaagtgacagtgtcttgccgttgttaccatatcaagtcttggtttatctttctttcactaattatttgcaatttaggaatacttttctaaattaatgagtttcctgtttaagttttttttttttttttttttttgattacaattgctataagcttggttgttttaacatttctttatttctgttttgcaatgagtcttttgaaagttgaaactccaatccccaaatcatcaagaaaggaaaagtacaaatagctctgagtccattttcttatttataaaggtgagaaaccatgtaatctaataagtaaaataatatatagtacaacactagtagactcttagaagcagcggcaatgcaaaagtttggatcagtatgtgtttcttggcaaaaccagcagccatacccgcgtcaacccgcacctgccctgcaaccgcaagttttttttaaaaaacaaaattccacccgccccgcttaggttcaaacccgccccgccccgtaccgctctattgccatccctacttctctgagttggcttgggccaatgtaaggaaaccatagctagtccaactatgctctacgtagaaatgactctaggtagtcattttaaagggatgttatttaaaaattaaccagtgcgtcctgaattttagtttttcagttcattttttcgggacaaaaatatcctgaattgtcctatagttaaggtatttaatttaaaatttcaagtcaaaataagtattgactaatctctaaatagcatccctgagaatgactatctgtacaattgtccctgagaatgacttggtgtaacacggatactgtggataaaatctcgagtacagatcgaaatttgttgaataatgggttactttataatattttcgcttaaatattaaacttttgtctatgatagcactcgaagtgtgacgttaatctcgatagcagtggtgatgtgtatgttattgataagctttacattttgagctga

SEQ ID NO: 7 - protein, 300 aa, Nicotiana tabacum
MFSGFSHFSCDAINACWAAPVLISLNIALKCVKKQSLSTEAIEERLAGVPVYALSNASEEFVLVSGVSTGKNLGLFCFSEADAEALRQQMESMDPTMRNGSRVVPVALNKVFQLKVDGVAFRLIPEASQVKNAMKERERTGTSDESFYGVPVFQSRSLILRSQNKRYRPVFFRKEDLENSLVRASQQQGRLNPALKGDIQVAVLEDIIQGMKDTSTSKWDDVVFVPPGFDVSTDPSQNNFDYALGPVMRQILIETGAKISEVFDNCRQILCAINFSHSKCDVNLDSSGDVYVIDKLYILS

SEQ ID NO: 8 - DNA, 881 bp, Artificial Sequence
  synthetically-generated oligonucleotide
agggatccaaaaaaaacatgaatatcttcaaacctaaacagtcatcttcttcttcagcaacaccaccacatctacagctccaacaaactttcaagaatttacaaacccatttctccaatttccttcaaaccacttttccgcaactcaacacactcaattcttctcaaaattcacaaaacccatgggctaaaattggtgttaataataataatagtgtaaaaaagcaatctttatctactgaagctattgaagagcggttagctggagtacctgtttatgcacttagcaatgcttctgaagaattcgtgcttgtttcgggtgttagtactggtaaaaatcttgggttattttgctttagtgaagctgatgctgaagctcttcgtcagcaaatggaatctatggaccctactatgcgaaatggctcgagggttgttcctgttgctcttaataaggttttccagctcaaagttgatggagtggcttttaggctgataccagaggcatctcaagtaaagaatgcaatgaaggaaagggaaaggactggaacgtctgatgagagcttttatggtgttccagtgtttcagtcaaggagcttaattctgaggagccagaacaagagatatcgccctgttttcttcaggaaggaggacctagagaattcactagtaagagcttctcaacagcaaggccgattgaatcctgctttgaaaggagatattcaggttgctgttctggaggatataatacaaggcatgaaggatacttcgacgtcaaagtgggacgatgttgtatttgttcctccgggtttcgatgtttcaacagatccttcccagaagtaagagaacctatgtcaagtcatctcatggtgcttggtctagact

SEQ ID NO: 9 - DNA, 1491 bp, Nicotiana tabacum
atggttctgtccaagacagcgtcggaaagtgacgtctccatccactccactttcgcttcccgatatgttcgaacttctcttcccaggtttaagatgccagagaattctataccaaaagaagcagcatatcaaatcataaatgatgagcttatgttagatggaaatccaaggctaaatttagcatcttttgtgacaacatggatggaaccagagtgtaataagttaatgatggattccattaacaagaactacgttgacatggatgaataccctgtaaccactgagcttcagaatcgatgtgtaaatatgatagctcatttgtttaacgcaccacttggagatggagagactgcagttggagttggaactgttggatcctctgaggctattatgcttgctggattagccttcaagagaaaatggcaaaataaaatgaaagcccaagggaagccctgtgacaagcccaatattgtcactggtgccaatgtccaggtgtgttgggagaaatttgcaaggtattttgaagtggagttgaaagaagtaaaattgagtgatggatactatgtgatggaccctgagaaagctgtggaaatggtggatgagaatacaatttgtgtagctgctatcttgggttccactctcaatggtgaatttgaagatgttaagcgcttgaatgacctcttgattgagaagaacaaagaaaccgggtgggacactccaattcatgtggatgcagcaagtggtggattcattgcaccattcctttatcctgagcttgaatgggattttagattaccattggtgaagagtattaatgtgagtggtcacaaatatggtcttgtctatgctggtattggttgggccatttggaggaataaggaagacttgcctgatgaacttattttccacattaattatcttggtgctgatcaacctactttcactctcaacttctctaaaggttctagccaagtaattgctcaatattaccaacttattcgcttgggttttgagggttacaagaatgttatggagaattgtcaagaaaatgcaagggtactaagagaaggacttgaaaaaagtggaagattcaatataatctccaaagaaattggagttccattagtagctttctctcttaaagacaacagtcaacacaatgagttcgaaatttctgaaactcttagaagatttggatggattattcctgcatatactatgccaccaaatgctcaacatgtcacagttctcagagttgttattagagaagatttctcccgtacactcgcggagcgactggtgatagacattgaaaaagtcctccacgagctagacacacttccggcgagggtcaacgctaagctcgccgtggccgaggcgaatggcagcggcgtgcataagaaaacagatagagaagtgcagctggagattactgctgcatggaagaaatttgttgctgataagaagaagaagactaatggagtttgttaa

SEQ ID NO: 10 - DNA, 12936 bp, Nicotiana tabacum
atggttctgtccaagacagcgtcggaaagtgacgtctccatccactccactttcgcttcccgatatgttcgaacttctcttcccaggtacatataatatgtctcaatcttaaataagttagagttaatttacgtcgtaaattcttttattccattctgcttaaagaatttatatatttttcaaaaaaaatttgatattttttgttgtttgattgtcagaaaaagattatttgaggaatatagggaaaagtcatttttcttacttttaacttcagatcattgtgttgatcaacatttagacgttactatcaatatttaatactcataatttcaccagaatgctattaatttgcttatattattattaaccattgatctttcacccaatcaaacactaatttttttctttcagaaaataagtccattttccgagaaacattttctgaaaaataactttcgtcgtactaaacacacccatcatcgctgttgttactatgcttcttttcatttaatattgagctgaggatctttggaaatggcctctctacctttacgaggtaggagtaagatctgcgtacacactatcctcctcacaccccacttgtggaatttcactacatatgttgttgtcgtaaactaaacacacccatcatcgctgttgttactgtgcttcttttcatttttcattgagccgagagtcttcgaaaacagtctctctaccttcacgaggtaccctcgtcagatcccacctgtgagattttactggatattgactaaactcacccatcatcacttgcgctttcttttcctaagattttcttttgtataatcttgaaaatggagtttctttttgaacttttttcttttgattttttggatttttaggtttaagatgccagagaattctataccaaaagaagcagcatatcaaatcataaatgatgagcttatgttagatggaaatccaaggctaaatttagcatcttttgtgacaacatggatggaaccagagtgtaataagttaatgatggattccattaacaagaactacgttgacatggatgaataccctgtaaccactgagcttcaggcaagtctctctctcttttctggattgttgtgacggagacagaatttctgctaaaggggtaaaaaaaaaaaatttaaaagaaattgtgaccggtagaatgtatcaaggggatttaaaatataaactataatcggattttattttgtattatacagtgcaatttttttggtgaagagggttcgagttccgccccctaaattcgtccttggctgatcgtgttaaaaatattatacacggtcaagtaacttataatagaatttaacttatatacatcaatagtgtaaaaaatatatttacaattaaactttgagatcagtgatcttgaaaataaaataagtttattacaaaagataaaggtgatgtgacagtgtgtgaagaatttttagtgtttgtatatattagtttagctcaaaattataaataaatatatataaaagtaataatttgataaaaatgatactccttaatttactgatttgtaaaagatcttttatactgtcgtcaatgtgtattcttctttctcgtattctttggtaataataactgataaaatggtaattaaaacttctaagctaaattacacaaatttgtaaaagatattttacaccgaaaatatatactagtataacttgaatcttcattttcgttttctttggtaataatagtagaatgccttgttgtgacttttgcgtcacaaaaagaagaaaaatagtactgttaggtttattctggaatttattcatctctcaatgaaacttttctcaaattcaacaaagtgtgtggaacagtaaaatgtccccaaaaatatctaactttttttctacttttaagtgtagcgtaggagaataaacaatgggcaaataacaaatttaagtggtactcaagcatcataggcccacgtctttttttttttttgttccaatacatgcaataatgcaaatcatgtccttgatataagtactataaataaaatatcttgggactcccataaacttgacacaggggcgaagtcggaattttaagtttatggatttaaaatttcaatccttttaagttactgcgttctagttaataatttataaatattcaatcgattttttaagtcaaacaaaaattttggaccaaaactactgaaatcgatgcatacgctcttattccaaacacccatccaaaaaaaaagaaagacaaaaaagaaacatgccatatatataagttattagtacttcctccgtccaagttttcttgtccactataaaaaatagatatcaattgttatttatccagttcaaaaaatcaatggataatttactattttatacctattttacccttgttattaagtattagtacttatttccaattcattttcaatatataataaataggagtaatatagtaaaattattatgttatttattattttttaagacgtgtgtcgagtcaataatagacaagtaaaattggacggatagaataataaacatctattgcattttgctcatcccctaccacctgtctttgttctactttagtaaaagatctttcactttactatagcatgaaccttgctaatctttttcacggttgatagtgtaaaacaataaaagttacacctttccctcccaccaaaaatataaaataaacattgattaaaaactaagggtccaacaaaaaatataaaataaacactgattaaaactaaaggaaaaacaaacataaatgtagatccctaaatcttggaaagctttaactaaatgctccataatcttcgatctcgatactttttaatgagttttaataaatctttccgcgtctagtagcagctcctacacattttccaaatattaaaaacaaaaagggttaggtttagaaagaggaaaaagaaagatatggaccacctgagtagaaactgattcggaatttaaatttaatcgattcaatttttgaaattattaacactaaacttattatactttaaataatgtgttcaaatttaatatttattgaatattaatggttttcacatctcaatttaaattttgtgacaaaaataataaattcagttgcactcgttgctaaaataataataaaaatgacaaagatggttggacttgttcctcctttttttttttgggggcaccatagagagagttgtacttatttttctccattttgagattttttttttaattattatctcaatatttcagatagggacatcctttaaaatggacaaattgtggggtaatggaaaaataatgttgtttcctttaatttgtttttttccttatggtttactttaccgacatatacgatggcttttgccattcttctttgggtggtaatattagttttttaaaagcgagtttaaattaaatattaatagttatttttgtaggcgattgcaagtagtttaattttaattttaattttatggtacttaaaaagaccttaaaaaagaaagttgaagtttaggatttccatttttcctttaaaaaggaatattctagaagcattacagtcgacgtaaaaaaatattactcccttcggtccacaataagtgattttttggcttttattatggtccaaaataagtgatttttccagatttcaagaatgaattaattatttgtttcctacattgccgttggagtcaatagtgttggagtatggtatgagtgtttatgtgaagagatagtaaatgttaatatgatcaattttattgctaattaatattaaaaggtgaatttcttaatcagtgcgaaaacagtcgaaaaatcccttattatggaccggagagagtattaataagcaactgttttgtctaatttggcagttgatttgtttaaactagactatgattttgtgaagtttaaagtcgttttcgatctgtttgaatttgtttctcaacctagctagacgaactagtctaacaaatgtcccataattatatttaaaaaaaaaattccagaaagtctgattttttgttattaaagaaaagtcaattagtgactcctggccccaccacgcaaagagttcaaatttctgaaaatttgattagtttagttaatgcataaattaattaatgcataaattttgacgggggatttaaactaaagtgaatgaatgaccatatgccacaattttttaagcagatattttttcctattaccattttatccttcactctgtgctattactccctctatctcatattatgtgtcgtgtttttttattacacgcctcttaagaaatattaattaggaaagggattggactattctacccttatttatgtcttaagatataatttatcttcattgaatatttattctatttatattttatcttcatcttcaagaacaattattactaagggtaaaaaaggaaaaaaatatcaattttgtcttgaacttctaaaatgataaataatttgagacaattatttttagtaaccatgactgttaatatgagacgaagggtgtatagcataggactttctaccacctgtgatcttatatcccctttacatattatgtaaactcataaattgtttaataacattattattttaatttaagttatagcccctttacatattattttattatgcatttttatggtactaatatatcggctcctgttgctttttttgagccgaaggtctcctggaaacagcctctctacccttcggggtaggggtaaggtctgcgtacatattaccctcctcataccccacctgtgagattataccgggttgttgttgttgttgttatatatacatcaatactgaacaaaaattttacaccttcaggccagatttatctattgtagcaagtatattgacttatttttatattgcaaatttcacactaaaaggaagcttacctacaaatattctttgggagtatgagtgacgtgataatgaaaaattttcacagacgatgtatataacttaaaatcaaaaattatatcgacaaactaagaatacgtttaatttgtcagaattaaataattttaaatctttttatttttttattttattttgcagaatcgatgtgtaaatatgatagctcatttgtttaacgcaccacttggagatggagagactgcagttggagttggaactgttggatcctctgaggctattatgcttgctggattagccttcaagagaaaatggcaaaataaaatgaaagcccaagggaagccctgtgacaagcccaatattgtcactggtgccaatgtccaggtaagataaatctatatttttagccgctcctaaaaattaataaccgacgaaatatatatttgttggtatgcatgtattatatacatatctagtaaatgcaattagtttcagccgatcggttaattttgtattttggccaatgttagcctatcatggatctttacacaaatagccgattgaattcattatttaattttgaaatttttacacaaataagcggatatattaactatttactttttctatgtatatatacattgattatatataattatacacatataatgttgttccttctgtatcctctacttgtaaataatgattttggaaattagaacgttagcttataaacgtaaatataaataaaacagaaattaattcgagcccactgaattcacagtgtttccttaaggaatttagtcccctcctagtacccaaggttatggattatttcctcccaggatagaacgaattacacactggtgtagcggtacttcaaaccccagtgtttcagcgaacacaaagttccgcagcaaatcacacttatggatgctttgtttgtagttaaaaataatgcagaataaggaggacagtcgaatggaaattctgagaggaaggaatgcaaagtatagccaatgttgaattcttactgaagagaatatcagattgcaattcgtttttccagtgtatacgcagtgtatacagagtgtatatccagtatatacagagtgtatatttagtgtatacagagtgttttgagtgttttttccgatgtgttcttctttctctccaacttatgctctatttatagcagttatttgagagaaatccgcccctccatggtgcaaaggtgtttggcaaaggtgcaagttcctaaacccaaaggaccgaaaacagttgattgtgttttcataggatatgcgactaatagtaaagcatatcgatttctggttcataaatcagaaaatcccgacattcataataatacggttatagaatcagataatgctgagttctttgaaaatatatatccgtataaaaaggaatgtgagtcgattggtgaaggatctaaacgacttcgggaagaaacaaaagaaagtacatttaatcagggggatccaagacgtagtaaacgtcaaagaacgtctacttcgtttggaccagattgtggtgcaaattggatcaccggttcaactgattcgaagtccacaagtggatatgtattcactattggtggaggagcggtatcttggaagtcgtccaaacaaacatgtattgcccgctctacaatggaggctgagttcatagccttaaataaagccggtgaagaagcttaatggctccggaatttcttggaagacattccattttggcctaaatcgttggcaccaatatgcatacattatgatagccaaacaacaattggaagggctgggagcgttatgtataatggtaaatctcgtcatatacggcgaagacataaaaccgttaggcaacttttctctagaggaattatcacaattgactatgtaaagtcaagtgataatgtgtcggatccacttacaaaaggcctaactagagaggtagttgagaaatcatcgaggggaatgggactatggccgagaacaagtcattgtggcggtaactctacctagaagactggagatcccaagatctaggttcaaggagatcaaacaaagtcattaatgacggttcaacattgtcaacaaatatttttagtccattctcgtgatgagacaatgttcagtaccaaggataaaacattaaggctttttaatgatttctaaatttaatacaaggtatatcaaatagtgtatctaagggatgacacgtttaggaatcacctatgtaagtgtgaagtattagccgcttcaatgagaattttgcaaggccaattccctacgcacttatgaaaccaggcggtgttcatggctgaaacgaacacaacaatgagaaccaaagacggttaagggattgattgtgtgacttatggttgtctaggtatacactaaagttcgacggttcaaagatatcaaatctaccgattgaccgagtatatccgacataagttcactacggaaagttcaaagggaaacctacttatccagatgcaattaatccttgtttgcaaattacacaagtttttcatgcatacttccgtgatatagccattccccattcatgtgggggattgttgagtttttgtttaagatgaaatagtcttaaaattagagtgaatggaaaatgggatttggatttggatttggattcggatttggtcaaatgatcgatcgattgattaattttttggaccaaatttatttgttaatagtgaatattaacgtgatataatccgtgtttgtaacggatgttttccaatccgtgtattgtattgcaacactaagcaataagcagcctagtgcacctcccacaatggtgcaagtgctcctcccaccaagcaagtgtacattccaccatgtaagtatttactccatgatagcctactgcttgttgcaccatggagggggaggatttctctcaaataactactataaatagagcataagttggagagaaagaagaacatatcggaaaaaaacactcgaaacactctgtatatacttaatatacactctgtatacactggatattcactctgtatatattggatatacactctgtatacactgcgtatacactggaaaaataaattgcaatctgatattctttttagtaagaattcaacattggctatactttgcattcctttctctcagaattttcattaaattccttaagcttgttgttccttctgtatcctgtacttgtaaataatgattctggaaattagaacgttagcttataaacgtaaatataaataaaacacaaattaattcgagcccactgaattcatagtgtttccttaaggaatttaatcccctcctagtacccaaggttatggattatttcctcccgaattacacactggtgtagcggtacttcaaaccccagtgtttcagcgaacacaaagttccgcagcaaatcacacttatggatgctttgtttgtagttaaaaataatgcagaataaggaggacaactcagaagtcgaatggaaattctgagaggaaggaatacaaagtatagccaatgttgaattcttactgaagagaatatcagattgcaattcgtttttccagtgtatacgcagtgtatatgaagtgtatatccagtatatacagagtgtatatccagtgtatatagagtgtatattaagtgtatacagagtgtttcgagtgttttttccaatgtgttcttctttctctccaacttatgttctatttatagcagttatttgagagaaatacgccccctccatggtgaaacaagcactaggctatcatggaggaagcacttacatggtggaatgtacacttgcttggtgggaggagcacttgcaccattgtgggaggtgcactaggctgcttattgcttagtgttgcagcacaatacacggattggaaaacatccgttacaaacacggattatatcacgttaatattcactattaacaaataaatttggtccaaaaaattatcaatcgatcgatcatttgacaaaatccaaatccaaattccatttctcattcactctaattttaaaactatttcatcttaaacaaaaactcaacataataatacataaattatgcatgtattatctattcagcggttattgttaatttaaatggtagggtggtcggctatttgggctaattcttctttacttttcttagctgatatacatagattatacattaattatacaaatttttacatccgatgcaatcagtttaaacggctaggtggatggctatttagattaaaactcctctaattttattaaatataaatcatttttgttaccataagtgtatttaatatgttgtgatagataatatatcttactttctaggctactaattcaattttttatggactgtcacctgtatttatcttttatagcctgtttggccaagtttctttttggccaaaagttttttttttttttttgccaaaagcacttttagccaaaaattgaggtgtttggccaagcttttagaaggaaaaaagtgtttttgaggagaagcataagcagttttggagaagcagaaaaaagtatcttctctccaaaagcacttttttgagaagcactttggagaaaaatacatttagaagcagttttttaaagctgggtcaaacactaattgctgctcaaaagtgcttttcaaactaattagccaaacacaaactgcttctcaccaaaattacgtttgagaaaagcacttttgaaaaaaacacttctcaaaataagctgatttttgcagtttggccaaacgtttaaatttttttgcactatcgtgtagagaagttaaactctataaaacacatggatttgtttccaaaatttaggaattgagagtgctaattttgtaattttaacaggtgtgttgggagaaatttgcaaggtattttgaagtggagttgaaagaagtaaaattgagtgatggatactatgtgatggaccctgagaaagctgtggaaatggtggatgagaatacaatttgtgtagctgctatcttgggttccactctcaatggtgaatttgaagatgttaagcgcttgaatgacctcttgattgagaagaacaaagaaaccgggtaagtcacgatttcgtagagctttttggttgttaagttatagtgtcgaccgaataatatccaataattccgacctttctggtcaatggtgaatacgtgtttgttcaaatatctttttttttttccttctctttgtatgaatatcacaatagaaggggagtcttggagcaacagtaaagttatctccgtgtgatctacagatcacgggttcgagctatgaaaacaaccactaatgtctgtattaggataggttgtctacatcacaccctttgtggtgcgattcttccccgaaccctgcgtgaatacggaatactttatgcaccgagctgcttttttatatatgtaaatatcataatatatagttgataatttgtaacaggtgggacactccaattcatgtggatgcagcaagtggtggattcattgcaccattcctttatcctgagcttgaatgggattttagattaccattggtgaagagtattaatgtgagtggtcacaaatatggtcttgtctatgctggtattggttgggccatttggaggaataaggaagacttgcctgatgaacttattttccacattaattatcttggtgctgatcaacctactttcactctcaacttctctaaaggtataattccttcattacaagtccttaaatatgtgcttaatccaaggcgaactaggatttgaggttaatgagttatggacttgtcatcaaatccataactcgtcaaaatcgagttcggatgatgccattctctttttctgaaggggaactttagagcaacgataaagttgtctctatgtgacttataggtcacgggtttgggccatgtaagatgccgctaatgcttgcattaaggtcagttgtttatattacattccttggggtatggtccttccgcaaaccctatgtgaatgcatgatgctttatgcaccaagctgccttttactatcataaaacatatgatgctctaattagctagatatatatatttctaaggctaaacattgaaaagtaccactagagtcatatcactagccttacaaatctaatcatttttgctattgtaatgcaggttctagccaagtaattgctcaatattaccaacttattcgcttgggttttgaggtaagttaagattaattttgttattttcaatggagctatgggcaggcaattgctatcattacttctaagttctattagtacaatttaatcaactatcaattgcataaaaatacgagtttaaattatatacatcatcattctaactaatttttacactatcatattacttttatgtgttatatcaagtaaccagtcttaatttaaagattacaaatctcgcattttatggtgtctagcctatggatatcttttgaatgacctgatgtaagaaacttgaactctaaaaataatatctttttcacaaacaacacactttaaatatactctttacaatctgaaatttccgaaagtgaagcctcggcgtaactggtaatgttgctacaatgtgaccagaaggtcacgggttcgatccgtaaaaacagactcttgtagaaatacagggtaaggctgcctacaataggctcttgtggtccggccctttccccgaccccacgcatatcgagagcttagtacattagatttttttttcttcacaatctgaaacttctatgttaaaacagggttacaagaatgttatggagaattgtcaagaaaatgcaagggtactaagagaaggacttgaaaaaagtggaagattcaatataatctccaaagaaattggagttccattagtagctttctctcttaaagacaacagtcaacacaatgagttcgaaatttctgaaactcttagaagatttggatggattattcctgcatatactatgccaccaaatgctcaacatgtcacagttctcagagttgttattagagaagatttctcccgtacactcgcggagcgactggtaagtatcgttacgcctcagttccaaataagttgaaattagactatataaatcgttacttcttcatttaaacgaaaagttgtgtcttacaatgaaaggacatttcaacccatgcaaaagttttaaaaaaaaagatattcttgtcttggcatctattatcaaaatatcttttttcttttcctccaaaaaacacttcttttctttccaaattatgtacttaaaaaaaaacttgaaatatgtcatgctttactaaccaaaactctccactatttcattagcacagaaatttgaaagacttgtcacttgttatatttactagaagaattaaccctaatagcagctcagtcgaccacttaaataaaaaataatcagtagatgaataatatatgcataattaatatacaaaggctatttgcattcaatccctttgtgtttttttaatcgtactttaaattttagtgggcgtttggacttaagaattgtaaaattccattaaaaaaaagtgaactttttttgaagtgaaaatgatttttaaaaattagagttgtgtttagatattaatataatttcggttgtttttgaattttttgtgagtgatccgagtaaaaaattttaaaaacagcctgttggagtttttcaaattttcgaaaaattctaaaatttatttttccgattcaacaggtgatagacattgaaaaagtcctccacgagctagacacacttccggcgagggtcaacgctaagctcgccgtggccgaggcgaatggcagcggcgtgcataagaaaacagatagagaagtgcagctggagattactgctgcatggaagaaatttgttgctgataagaagaagaagactaatggagtttgttaa

SEQ ID NO: 11 - protein, 496 aa, Nicotiana tabacum
MVLSKTASESDVSIHSTFASRYVRTSLPRFKMPENSIPKEAAYQIINDELMLDGNPRLNLASFVTTWMEPECNKLMMDSINKNYVDMDEYPVTTELQNRCVNMIAHLFNAPLGDGETAVGVGTVGSSEAIMLAGLAFKRKWQNKMKAQGKPCDKPNIVTGANVQVCWEKFARYFEVELKEVKLSDGYYVMDPEKAVEMVDENTICVAAILGSTLNGEFEDVKRLNDLLIEKNKETGWDTPIHVDAASGGFIAPFLYPELEWDFRLPLVKSINVSGHKYGLVYAGIGWAIWRNKEDLPDELIFHINYLGADQPTFTLNFSKGSSQVIAQYYQLIRLGFEGYKNVMENCQENARVLREGLEKSGRFNIISKEIGVPLVAFSLKDNSQHNEFEISETLRRFGWIIPAYTMPPNAQHVTVLRVVIREDFSRTLAERLVIDIEKVLHELDTLPARVNAKLAVAEANGSGVHKKTDREVQLEITAAWKKFVADKKKKTNGVC

SEQ ID NO: 12 - DNA, 526 bp, Artificial Sequence
  synthetically-generated oligonucleotide
aattggatccgagttgaaagaagtaaaattgagtgatggatactatgtgatggaccctgagaaagctgtggaaatggtggatgagaataccatttgtgttgctgctatcttaggttcaacactcaatggtgaatttgaagatgttaagcgtttgaatgaccttttgattgagaagaacaaagaaacctaataagatcttcaacacctacaccatttttttaatcactactacccattgcattgaacaaacttccaagttcttcttagcttcagattaagaaagtaccctttcttggctttgttgatgtggtaccattgtccattgtcttgtgtgtttccggtttctttgttcttctcaatcaaaaggtcattcaaacgcttaacatcttcaaattcaccattgagtgttgaacctaagatagcagcaacacaaatggtattctcatccaccatttccacagctttctcagggtccatcacatagtatccatcactcaattttacttctttcaactctctagaaatt

SEQ ID NO: 13 - DNA, 708 bp, Nicotiana tabacum
atggggagaggaaaaattgtgattcaaaggattgacaatacaacaagcaggcaagtgactttctcaaagagaagaaatgggctgctgaagaaggctaaagagctagcaattctttgtgatgctgaagttggactcattattttctccagcactggaaaactctatgaattttccagcaacagcatgagggctataattgatagatacaacgagatgaaggaggagcatcataacctcatgagtcctatgtcagaggtcaagttttggcaaagggaaatagcaagtttgaggcaacaactacattacttgcaagaaaatcacaggcagcttctgggtgaagaactttctggactcagcatcaaagatctaacaaatcttgaaaaccaacttgaaatgagtttgaaaggcgttcgaaagcaaaaggagcagattttgactgatgaaatcagagaactaaatcagaagggcaatcttattcatcaagaaaatatagaactctataaaaaggtaaacctcattcgacaagagaatacagaattgaagaaaaaggtttctgagcaaggatgtggaagtgaaccaaatgggggtgttcaggccacacatgcaatcagcaaaggatatgatgtacatgcaccaatcagtctccagctaagccagccacaaacacagaagagtgtaacatcaacaagcgtcatgcagcttgggtaa

SEQ ID NO: 14 - DNA, 15537 bp, Nicotiana tabacum
atggggagaggaaaaattgtgattcaaaggattgacaatacaacaagcaggcaagtgactttctcaaagagaagaaatgggctgctgaagaaggctaaagagctagcaattctttgtgatgctgaagttggactcattattttctccagcactggaaaactctatgaattttccagcaacaggttagttatttttacatttttaattttaattttaatttggtcctaaacatagagatatataatttttgcattcttccttttttttttcctttttctttgggaaaagtttggactgaaatatgggattttttcctgctgtagaactgcctctatttcatatattctgtacttcttgcatatcgttttatgtaatttttttgtttaaaaattaccaatttggtacctttccatttactgctattttttattaaaaattattaccaagttggtatctttccagtttgtactttgtatgtgaaaaaagagtagtcagatcatatcatggattaacctttgttactgcatcaagattccaacgtgcatatttataaatgcatgctacgttactttcagttgttttttcttttcttttttttttccaagtatattgggagaaatctaaaactagctttgcttttttaatccagggattaaatttgttaatcatgcacgaggtgttttatctagcctggcccattctatacaaacctaattaatgttgaaaaaatgactcgaggaacaacatgcaccaatcctaaagaaaacctaataggagtagtaatatttgcaaatctgaaatctgtccgcactttagaatttggtttaaagccctgcagtgataaatatctctattgtattctatttggtgcaagtaagaaataactctttagagcacgtttggatgggaaacatgttataccatcattaattattccggaattagttatcccgagattagttatttacccttacaatagggataaacaaacactacaaatctacaaccccgggataattatcccaggattaattatcccatatccctcgatattgttattctctcttcagtcttcacataaaccctaaggtgtcatttggtttaatgattagaataaaggcatatgagatttaatacaattcgtgtccttgatcttattgagttaatcccacatcagtgaatgcaaacattattatgctgccaaatatattattctactaaactaacaaacaggatgctccttaattctacgtatgcatccagaaacttctgtcactcttttgtggccctcagataaactcacataagtagcttctcacataattagaatactttgtactacctttctatacaaccttctttagacgcatgcataatttacattagaacttttaatcttttcatcaagatatacttgtgatcactttaattatgtgtatattttgcttcgaaattgcctaaatagaatttcgtcttatggaatatagactcacaagtgcagaatcatacgtatagtttaatatggggctcagataactagtttaacacatgaatttgactcatacactaacaatgtaacaatttataagctgttagtgtattttggcgagttacctgtcttattactcctacttattatgcatcatggataattacctataattatcttttaggtgatttgataatgtaaagtttaaattcattatgttagtgtgagaagttaaactcttgacacaattatatatttgctatgttaccagcatgagggctataattgatagatacaacgagatgaaggaggagcatcataacctcatgagtcctatgtcagaggtcaaggtatagctctttaattatatttaaatctgcttcagaattgcctaaatagaattcgtttgatggaataatggacttgcaaaggtagaatcatatgtatagtttaatttggcacacagataactagtttaacacaggaatttaactcatacatatacattggttatatacataaacaccaccgatttttgttttcacaagtggttgttaatagagaattgcgagtgtatgtaatgtccctttttggatgttcttgtatactagactagatgtgttacatcgtactcaataccttgtgagaagggatttaggaaaagtctgctctcattctatgtcagagaatctaaacttccaattaaaaatctttaagataatggattaaatattctttgctatttaaccttttaaatgatcttgtatatccattgtgggatatatatatattgagtaactcatcaaatgtggagcagataggctcgaactaaatgttatagttggaaattttcaggttattattcttatccttcaaccacgcgtgtggacctctatgggaaacattatctatttaatttttcattttggttagctcaaatatattctgtcgaaatctcaatcaaagatagtataaggccagaatttgaaagatgattcattttttaaagttccacgtgatatctttataagctaaatatgaatgatgcaagctttcagtcaaagagattgaaacagtcattaatcaactatggcacccctaagattgacctcttttttaaatgaacctcttaccctggcctcaacaatagcttttgagaaaattgattgctaaatgatttcatattactttatgttacaattaattgacaagtactttgattaaacagtaaatcggcgaaggatcagattagccacaatgacatcgacaatttttttcttaacagtgctgtaacagagaagcccagaaagagcacttatagtctccattatagaacaagagctacaccattctgtttgacaatagttgatgatggcaagttagctgtagcttcatttcccttttgaggtaggaattgtataaaaggcttggaattgtaaaaatacaaaaatttaaaaatgcaaattaatggagagttgactaactcccaaaaatagattgctatggagagagaacagatgtgaataatagctcttgatcttcacacatggtcaaggtgcgactagattaaagcaaatacaaattcttcaagaacaacaaaaggtttttaagcaggttttttcaagcaagctcagttgaaggctcacagtggagtttagggagggtcaaaaaagttttcatgatgatcaaggtcatcctttggcccaaactaactccatattatgttatcagccttttcccattcctttattctcgagttcaccccgtctttatcatggctcacggaagtcttgcaaaaagtttcaagaccgcaggatccacctatgtgaatttcgtgtatgcattaagaattcagtaacagtaggcattcatctgaagtggctgctctttctgggcatcttgccccattcaaacttttagctatgttagcgtggtcagtgttcttcctctggcgccaaggatggctaggaaataccaatggaacacctgaactgggacaatccacccaccaggttttggttggtatatgtcagattcgttaactgactccatggtaacttctggtaggtatcttctcaacatggttatgagagagattcaacttactagaaaaacagaacacgatattagagagccaaacagtcagaaaagttaatgacatatagcaaaagctaaaacacgaaatgtaaatcagcaaactcatagagaaaggataaacagaatctttgctgtgcaccttagtgactgggtgaggagggggaataatcctcactttgttgatgttctggttgtttttgctgcctttactgcttcatttttcctctctgcctgctggggaatttcatcaacttttttttttattaaaaaaagctacccattataagacttcacacattcttgtggtgcaatgctacacttctggaaacttccatgtgttggttggtactcttttatctttttccacttccatactcttcttgtacatcctctcatgtatcttcttccatggttctgctatcttcttgttattctcctttgccctcttattcctgcttattaattgttggctgattccctgaatagatgcctatcttgttgtcccttttttccttctccccctacttcatgttcggttcttatgcttgctcgagacaacaacctgcttcctcctaattggtcacttcaagcatcgatagttaccattgactgttaaccttcttccaatgcaaatatatctgactcattagttctatctatgatgtgttgtcaattgatgttgatgagatggtttagtaaacataaagggggatggagtccctgttggaggtgtttgtgttgaaaggcctctagtatcattccctcgcgctataatccctctccctgttccttaatctaggaagctcgataaaccttgggattaactccagtcaaatacttgattcctgttctttccttggagcagttcgatcaagtggaatcaaatcctacaggctcatatgctaacactgccactcagttactctataagatttctataagcatgaagagaattttgtgtcaaatgctgtatctcatgacgatgtaaagaaagttaaatggtaagcttattttgaaaaggattttggaatcgtgctttgatcccaaaaggtgctgccttcctctattagggttaaagctttattagcacaaattgggacttctgttagggtttgttccggtgccaattaattcgtaattgtggcctattgtaacctaactacacgctcattcagagttccaaacaagttttactttatcaaatccaaggatcgattcttgaattgcaacacctacgctattatatgtcatactagtgaactactttgatggaacctaaacaaatacagtaagtcatctataatcatctataagatactgaaaacagaaacccaacctaaaataactaacaaggtctcttctcaaagttgagtgatccatagttacctccatgtttccactactaacctgaaaaatccatgagctgtgtagagaattcccttaaagcctccactacactctggttcctgtattgtctgcattacaaaatagcaggtttgaacctgtttcaggaagtttttcctaccctccttcccaatagtaagcatagtcccataagtgaaaggaagcaataagtatcaactcttaatcaagtggtaaatactatcatcttaagagttatccagcatgatagatacttattatccatctacataatataccacttatcatatttgaatcaggtcatcatctccagagacagttatagattctggctgatgcagcatttgttgttccaacaagttctatataagcagaaagccaaaccacaagaaataccatatcagatcaaacagatgcatgttggaaattggaatagtttatcccagacaaatagtgcaggaacaaactgataccggttctttttcccagtttatgttgcactagttttgagaccaaaagtcagccatcaaacagtcatgatgcctgaaataagggaggtcaccggagaataaggtggcgacaaaactagtaatgctcacccgttacagtttaattccactccaccatgtgcactgacaagagaatataacctaggggaatctgcctgcagatgagataattaggctaacaagcagaaggaatacgatggtcttgacatgataagccggagtttagagtttgtttatctctgcataagcagaatccatgatctaattaatcaactaaaccataatccaaaatcagttgaggccggctatatgttcctatatatccattctgctctgaaactgggatctaatgcctctttaatttgcatttgcagaaatgaagtgaaatcccaaaaagacatctgcaatgctaggttgaaggtccagatgagacactattttaacaaattccattagaggatagttcgtttgtctaacagagaatgctttaaaattgcagatccctatatcagaggagaggatggaggatgtctcaaccccacctaaatcgatataggatctactctcagaggtaagtaatataaaattttcaaaaaggaagtcattccacaaacacaaaatataaaaactcagttggatgaaatgtctacacaagtttagcgattgaaaaccctaccaaaggtcctacgtgacacattatgacaatttgctcaacatcgcaactatttatagattaaattagatggaaaacctaagtttgaattcctatccatggataccgtaattaaattataaagataaatagtcttccccatctagggagcatagttcatggagcaaattcatgtgataattcaacaaatggaacctaacatatctaataaataacctgaacctgagtgtcctggtcttctgtctcaaactagcatctattcctggtattgcatctcaaatatgaccaaatccttcactggtgctaaatcctacttttgtgctctcaagttagcatctattcccttcgttagtttacccactgtaactgacggtcacgtccaacgagagcgtgagcatcacactattctttcttctcatggaggcattctactagcaaagaagactcctataagtggtagcaccttgttggggctttgtggtataattctttgccgaaagaggtctctccagtgttgcatgtttatatctacgaccgatccctcaccagagctgacggacatctcaggtaaccatccttgacttaccgacatgtcaatgaggatagcaaaaaaggtatccaactgggaagaaggcagtgagggtataagtattatcagaaatttcaaatgacaagaaagtaaaagttcaggtgctccattaaatccaaatcatatatgtcaatgaccaagggcatgattaatcaaaacataccatggaatatggattcatggttttctaaggctggaggcaagcaaggacattaggaaaatcttgcaatgattcctgaagcagtcattccggttggaaaaaaacacccttgaggccttgaccatccgaggaggataacctgagagtaaatggacatgaacacagatgaaaatattcacatacatatcaagttcataatccatccacaggagttctctatattcctccaggacttcaatctcactacgaatccgtcattaaattgtcaatggtaaaagtttaaaaattgcatccttccagcctgaaagacaatatcaaccccaaccaatgtatgtgctatcttcagacgttcatcgctaaagagtttgtttcttattgctatggaaaaactgagacacgatacatttttgccgtacattgtttaccactagttgatctctattatcaaacacgggtgtcaagttccattttacctgttcaaaaaaagggtgtcaagtttcctatttagaaaattgggcagggagcctacaggtcgaagagatgcacaattacaatctcagagatccaactgtctaaagagttgacgcacaataggggtgtacaaatgaaaccgacaaaccgcaccaaccagataatccgagtcaaaccggaaaaaaaaaccgcctatagtttggtttgatttggtttggtgttggaaaaaaaaatccgaccatatttggtttagttttaactaaaaaaaagtcaaagcgaaaccaaaccaacccgacattatatgtgtagaagttttaaatatatttaatgcataaaaatatttattgtagtgtagtttataaatatttcttaaattttttcataattttatcttttaacgtattatttcaaacttgacttataatttttggatgctccaataaattttatagtccataaatgttagtaactcaaataaatcctaaaccaaaatcaaatcaatactaatgctaataaaaaacattcaattcaattgtactatgaatgaaaatagtgttggatatctatttttaagcttattcatgatttagataaaatgcataacttatttttcttttatagtgtttagtcatgtaaataatagtatatagtcgtaatttttaaattatgtttgttttcattatggcttattaataatatttattttgtgcaattttattatctttattattgaatattttagtacaatgccataactcatccaatatttatgttattttattgaaaaacaccttatatagttctgtcttactagattaaagaaatatttggagcaaaaattctatgttttgtgctatgaagactttatgaaaaaaatccggaaaacccgaaaatccgaaaaatccgagaaaaaacgagactaaaaaacctgacttttattggtttggtttggtttttagatttaacaatccgatacaattggtttggtttggtaattagaaaatccgaaccaactcgacctatgtacacccctaacgcacaacaatgcagatggagttcggggtgcttatcgggtggataaaattacgcttaacggttatcggattataaatgttgtaatccgctaaccatccaataagataatgggcagattggtatcgaattgacaattatcgggcagtttatcggctaaacaaaataaaaaacttttgaacaatcaagtacatacaagaactactgataaggaagacataacagatacgagctaatctatgctaaacatgaagaaaactagcttcctccatcttactacagatctacctaactttattgagctataatatgagccaacggtagaagttagggatttagagcctgtttggatgagctgatttgatgtacctgataagcattaggtgctgaaaaacacttttaagtcttgaaactgatttaataaataagcagttacgcgtttggatacaagtgctgaaattgataataagctgctacagtatttgataaaaaagtgctgataagctttttttctgttaaaatgacttaaataaccttataagtatttacacctataagggcgtaatatcttcagaattttagattccaaatcgatccaaatacaaaatattctatttgtcattttattttaaatacaactgtgcttcgataagataattttatgataaatataatttattttatgacaagcatataatcataagttataataattaataaattgataaaagtttctcagtaaaaaataaacctaaataggacaaaatatttgaagagaaacaaacactgtctttatcagcacaacacgtagaaagcaacataccaaaaatttgatatgtcctcatttattatatacaattcaaagattaatacacaaatcacatagatataaatatgcaaaggaatagagaatttgcttatcttaaatagtcaatgagcattgcagacttgaagaggcggagggagggggttaggttgaaatagtactcgaggcattgagtatcgatgcaaataacattatacgtgtttacacctataagggcgtaatatcttcaaaattttagattccaaatcgatccaaatacaaaatactctatttgtcattttattttaaatacaactatgcttagataagataacttttatgataaatataatttattttatgataagcatataatcataagttataataattaataaattgataaaagtttcttagtaaaaaataaacctaaataggacaaaatatttgaagagaaacaaacactgtctttatcagcacaacacttagaaagcaacataccaaaaatttgatatgtcctcatttattacatacaattcaaagattaatatacaaaccatatagatataaatatgcaaaggaatagagaatttgcttatcttaaatagtcaatgagcgttgcagacttgaagaggcggagggaggggtttaggttgaaatagtacttgaggcattgagtatcgatgcaagagttttgttctaaaaaagaatattttaaagataaaataataaaaattttggtcaaacttaaagtgcttataagctaaaaatttataagttgggggttactagcttacggcttattttttacttataagcacttggcttataagtacttttaactttaccaaacgcgtagataagctactttgaccagcttataagcttagccaaacaccctcttagccgtttagggtttcaatagtactttatatacataggggaaaaaatgtaaatataaaaattcttaacgggttaacggtttacccgataagaaatttgagtaatctgccccaaatcgttaagccgttaattataaaatctcaatctgttcaccatccattaccccgataatccgataccaataagccaataagccatcggtttggttggttaacggttttggtttgattttgaacagccctagatggtgtttttggctaagagattatttctacaaccaagctctgcattcgtaataaatgtttttttctccctgaagaccagggtccgcttggtacatggattgcgcatatgataggatatgtaacttcgtatgcatgtattctcgacaagattaattaactcaatctggtgaggacaagattattaattaggcaggtactcaatagagaatttgcttattacattctatataattcattgctcattattccacatagtcattcctagggcattaaacttcatagttacccgtgataatcacaggtccccaatagatgattagttgaccaaagatcccaaatgtctaaggtgctgaaagaccaagaatgcatatgtaaattttgtgagaagttaattcttaaaccatgttgagcaattgtaacagaggtttctttcttgcttcctgaagattagctgtcatttcttacacagactgctcacctgaaaaggtttacctcccccagtttttagctaggtacattaatcttaatcttaagagactagaaaactgatcggcagataactattaatctaggccagcaattagtataagaggcaaaaggttcaccatacaaatagaggataagcccttctttcatttcttttcctcaatctcctcctcttaatcctttcttccaggtccaacttctgctttccccaacccacccacccacacgtcagtccttgaccgtccacatgcacctttttccccccaacctttcccactatgcaatttcaaccctcaccccttgggaactaggggtgggcattggtcggttcggtttggttttgtagaagttcggtttagtttattcggttttcggtttgtgattttaataaccaaaaccaaatcataataacttcggtttggttcggtttattcatgttcgattcggtttttcggtttcaagccatggcaaaaatagtatgaaacaacgaaaatagattacttgtgagagaatagccaaaaagggtaaccaaaaacatattgagtgcttataaatattctccatttatttttgttagactgcattaatggtcatataatataatgaaattctatatatatccaatcagtgaaataagtgaatgattagcatgcgaattcagatgatacggaagaatgaattgtgcgaatgaggctttgtttatttttctgtagatcccattcacccgttactaaaattcaaatacgaagaaggattacatcaattccgcaatatccgttggggttaaaattcttgttgtattttatattgttcttaattcggttataaataattcggttttgggtttaggctaaaaaaattcggtttttcggtttaaccgaaaaccgaaccattaaaaccgaccaccgaactttttaaaactataaaccgcaaaccgaccgaataaaccgaaaaatcgaaaccgaataaaccgaaattttcggttcggccgattttttcggttcggttcggtcggtattatgcccacccctattaggaacccaattatttttgcctctccttaacatgatccttcttctttccttccatgacatcattccctcctccctccacccatccctaacattttacaaactatcgtggcattaaaagtatgaagcatgctatgaaattttggaaaagagcgatagatcataaacttacggacaccataaaagtaatgtagaaccattttggggtagatatacaacgaaggctatatgctaagaagattcatgaaaatttattgcaagaggaagaatctacacagcttagagaaagcgaatgagaagagtgccaagaaaagcttttggtgggtaatgaagaagaaaggaactcatattaaatatataatatcataaatgatatatgaaatagttgtcactagtgtgagaacagtagtacgagatacaaagagtttcccataaccatgtttttacacccagaataggcattgagccttgtttaccctacttatggatgagctaactcacactatatagtttgaggttacattgtacatgctattttcaaatggcattgtgctaattgacgaaaccatcaaggatatcaaccaaaacttgaacttctgatacgcactctaaaaagttgaagttttaggataagtaaaagtaagacatgcattacaagtttagcccgcataagaagagtgaagttgaggtcagaccaaacaagattgcaaggtttaaaagcaaccaattcatatatctaggcttgatgttcgaagagaacggcacaatagatggggatgttacacatccaatcaaaatagagtggtttaaatggacatttgctaccggagtattatgtaatagagggataactaccaaagtgaaatgcaaattctataaaacgattgtaagaccagcaatattacatacatgggagtaaatgtaggtctctaaaggctccaagtatccacaagataagtggcgcaaagatgaatgatcaagatccaaattcagatgaatgtatttactttctataaactttcaagttacgaaaaagtgctacatagataggtttgaacaaatgagaatagatatcgaggattcatatagttgagcccgtctagttttagattgaatcgtagttgaaacaaaactaagaacgttctacatctaatatgtggctctcatcatcctaaagtacttttcttgtatggttgaatttatcatgggttgcaataatcatcaagcactacaaagaaagatcaaagcaatatttacctgatttcatctcaggaattatttagccttctaatttcatcttctaagcactatacttatttttctttctttccttggttttggctagttttggcaaagggaaatagcaagtttgaggcaacaactacattacttgcaagaaaatcacaggtaaattgatttgacaaggtatatcttttacatgcctctttatgccacaggatcttttattgtacacactatagattgaacaatgtgatacctttatacactataaattgagtaatttgataccatttaatatattgacttgtgtgaaatttattatagggaatattttttagttaaatcttaatacgaccctcacgtgtcagtttttctttttctagtggatcgagtacataagaaatcattccatgaaggatagcgatgagactcgaattcaggattgtaaattgtcaaaactcaaaactacctcgcctgagttaactgctagggagcaaacatttatatttatttattctagttctccaagatagattgttaagtcattttttttttttgcctactttgtattcttataagtttctatgcataaaaaagttaaaaattttattggagataaagttttaagtaatatgagcacttgacaaatccaatcaacaatcaaacccattattacttttacttcatacacaaacaaatgccattttgggtaattaaccagaatttctaaaacatcatcaaaatttcttcatcatgtttccgaaaatagttatgatattttgaccaatcacatttttttatacaataatctacacctacttatccccagctgttgctggtgctttcagttgaatatgcaaggacttttaggggctcttttctagtgtttgaaacagtttaaggtttctcaaagcttcttttttttctttttttttttgagtaaggtgacaggtttctcaaagcttcctcttatcatagtctttacacttggggccatttaaggattggaaaacagaacaaaaaaggaaaaagatgctgcatactgattttgttttaaggttcatttctcacaagcattagagtaattcaggtttcttgaagcttttagtcaaatttatggtttagagcaaacactgggaaaacagaacaacacaaagatgccatgattatttaatttagaggttataagatacactcctagcatctcttgggcacaactgaagttaaaagtgcccaacagaactctaaaccgagtaaaataattttctacagctgaagttgctagcgattgattgctagtaataagaagaactataacaataaatgtagacaccaaaatttaactaaaaagccaaaaacctagtcaaactcaaatatcataaaattaagtcgatcaagaaagaacttgcaaaatgcccaaaaacaaaatttttaaaaaatctaaggattactaacgaaaaaagacatccaagacttgaatttgcaatgttttcttccatgtttttctgtgaacaactcctggaggagggaagaataactataaaaaatattaagatgaacatccccttcttttgtagcaacgtatcggagcttgtcggcatgcttaacatgcaattaaataacaataaaacgtgtatatttcaatgtctgagatctagcttagtaagctaagctgctaagggagaaatattttaactaatccctttcttttatgaaccacaggcagcttctgggtgaagaactttctggactcagcatcaaagatctaacaaatcttgaaaaccaacttgaaatgagtttgaaaggcgttcgaaagcaaaaggtaaaatccacacttttaaaattcttttgtggtcatgaaacttatgtttatatagtctacaacttatcctgaatgtattactttttcttgcaggagcagattttgactgatgaaatcagagaactaaatcagaaggttctactagaaaaaccatcagaacttcccatattctcttgtctttaaaattacccggatgattaatattgcttctgcagggcaatcttattcatcaagaaaatatagaactctataaaaaggtaaacctcattcgacaagagaatacagaattgaagaaaaaggtattaatttagagagtattgcctccacttgttgtttcaagatgtaccataaaattttgcttttacattttagtcttctaccacaagcatagatatccttgagaccttgaccttaatctaaaggagaagttacctatgccaggtttctgagcaaggatgtggaagtgaaccaaatgggggtgttcaggccacacatgcaatcagcaaaggatatgatgtacatgcaccaatcagtctccagctaagccagccacaaacacagaagagtgtaacatcaacaagcgtcatgcagcttgggtaa

SEQ ID NO: 15 - protein, 235 aa, Nicotiana tabacum
MGRGKIVIQRIDNTTSRQVTFSKRRNGLLKKAKELAILCDAEVGLIIFSSTGKLYEFSSNSMRAIIDRYNEMKEEHHNLMSPMSEVKFWQREIASLRQQLHYLQENHRQLLGEELSGLSIKDLTNLENQLEMSLKGVRKQKEQILTDEIRELNQKGNLIHQENIELYKKVNLIRQENTELKKKVSEQGCGSEPNGGVQATHAISKGYDVHAPISLQLSQPQTQKSVTSTSVMQLG

SEQ ID NO: 16 - DNA, 515 bp, Artificial Sequence
  synthetically-generated oligonucleotide
aattggatccatggggagaggaaaaattgtgattcaaaggattgacaatacaacaagcaggcaagtgactttctcaaagagaagaaatgggctgctgaagaaggctaaagagctagcaattctttgtgatgctgaagttggactcattattttctccagcactggaaaactctatgaattttaataagatcttcaacacctacaccatttttttaatcactactacccattgcattgaacaaacttccaagttcttcttagcttcagattaagaaagtaccctttcttggctttgttgatgtggtaccattgtccattgtcttgtgtgtttccaaaattcatagagttttccagtgctggagaaaataatgagtccaacttcagcatcacaaagaattgctagctctttagccttcttcagcagcccatttcttctctttgagaaagtcacttgcctgcttgttgtattgtcaatcctttgaatcacaatttttcctctccccattctagaaatt

SEQ ID NO: 17 - DNA, 1194 bp, Nicotiana tabacum
atgtctcaagatggctcagcagcagcaacaatggatcggaagaaggattctcaatcaacaacaaaccctacccgaaatggtaacggtaacggtaacggcggaacagcaacaaacggcgccgtttacccgtcactcaattctctgaggttgcgtttaaaccctagtattgatcacaagtcggataattatgaagatcttcaattggattttagtccattgttatttagctcgctcgaacggtaccttccgcctactctcctcaattcgtcacgtgaccataaagttcattacatgcgggaaattctccttaagtattgtcctgaaggtgaacgtacacgtgtgcagaagcatagggaataccgacagaagattatatcaaactatcagcctctacacagggagttatataccatgcatgctgcgaatttttttgtgccatcatttcttaaggcaattagcgagaacacagaggaaagttacagaaacataatgtcggaaccctctcctggagttttaacatttgaaatgcttcaaccacgattttgtgagatgatgttggctgaggtagaaaactttgaaaggtgggtccgcgagacaaagttcagaataatgcgtcccaatacaatgaacaaatttggtgccgttcttgatgactttggcctcgaaactatgcttgacaagttgatggaagatttcattcgtcccatttcaagagttttctttactgaagttggtggatccacacttgatagccatcacggttttgttgtcgagtatgggatggatagagatgttgacttgggttttcatgttgatgactcagaagtaactttaaatgtgtgcttgggtaagcaattctctggtggagagctgttcttccgtggagtgcggtgtgagaagcatgtaaatactgaaacacaacctgaggagatctttgattactcccatgtcacggggcgtgcagtgcttcatcgtggtcgccatcggcatggtgctagagcaacaacatcggggcagaggatcaacttgttgttgtggtgcagaagttctgtctttagagagctaaggaagtaccagaaagacttttccggctggtgtgcagagtgccagcgcgagaagaaggaaaggcaacgactgtccattgctgctactaaattggagctgctgaaaagagaaggggaagctgctacatag

SEQ ID NO: 18 - DNA, 5548 bp, Nicotiana tabacum
atgtctcaagatggctcagcagcagcaacaatggatcggaagaaggattctcaatcaacaacaaaccctacccgaaatggtaacggtaacggtaacggcggaacagcaacaaacggcgccgtttacccgtcactcaattctctgaggttgcgtttaaaccctagtattgatcacaagtcggataattatgaagatcttcaattggattttagtccattgttatttagctcgctcgaacggtaccttccgcctactctcctcaattcgtcacgtgaccataaagttcattacatgcgggaaattctccttaagtattgtcctgaaggtgaacgtacacgtgtaagtatagcattttcaattttgtaaattacatttttcaattttgcgtttgtaatttgcatgtgattgttgttgttctttgtacattttgattagtgtatatattatgttagaatgtgggtagtgaattgagccattattaactgatgagaagctgaaaagggaaaacttagaagctgaactttttctgtgctttgtattgcaattttgcatgtacgttgccattaagcaatttgctgaaaaatcaactttttttatgtcgaattagttttctcaatgaaacacctttgttagtattaaaaaatagtgaaagggtggcttgtggagctctaggtacgcagagctgtgaattcagctgtaatagagtgcttatatgctgtttgatgagaatgaaaaaaacaaaagaaaataaaaagctagaaaaatctgggctttttgatggttattgctgaaaatctcgggctttgttttattctcatccattattgtcctgaacgtgaatttgcattttgcacgtggttttttttttttgtattttttaccgtggtatctaggtcagcttgtgcgtacctctattattccaccggatacctgctacctccaccggcgcaggtactaggtagctctatccactaagacttaggcggatgagaaaaaatcatctaatattattttgcctccgctatgatttgaacctgatacttcgtgattctcctcccactgaccactaggccacacccttgggtgcgacatagcttgtttctcttttcaataggcaaatgatttaataattcagggagatgtgacccgagtatagatggatataagaacaaccaaaattttggttaaaaagaacatgtgatctaagttaaacctacctggttaatttgtttataatgtggtggaatatttacaaaacatgccagtctcctaatgaagtccttgtttacccttgaactattaggaatgttgtctgctgatatagtcttctctgaatgtcctttgctttccaaacttttccttgctatttgtgagattgtactctctctctctctctcattccgaaactctatcagtacaatattgtttcatctcctctgctttaacaggtgcagaagcatagggaataccgacagaagattatatcaaactatcaggtatttacgttctgcagaagggatttgtaggttaatatttcagtgatggttgtaaatgaagacatcaatttttatactttttgttgttaagtctattaaagtaaggtaagaaagtttacgtaactttgcttgcgttttctctggagagaaatgcctttccatttaaagaattataagcatagaatgtaatgctcattgatcttcgtttagcattaatcttcttcctttctattttctaattagctttccttttattccagcctctacacagggagttatataccatgcatgctgcgaatttttttgtgccatcatttcttaaggcaattagcgagaacacagaggaaagttacagaaacataatgtcggaaccctctcctggagttttaacatttgaaatgcttcaaccacgattttgtgagatgatgttggctgaggtatcaaccggcttgctgctgttattttgcatgctaaatctagtttttctttgtagtttagcatttctgttttcttatcaggttctattgcttaggtagaaaactttgaaaggtgggtccgcgagacaaagttcagaataatgcgtcccaatacaatgaacaaatttggtgccgttcttgatgactttggcctcgaaactatgcttgacaagttgatggaagatttcattcgtcccatttcaagaggtaagaattttacttttaactgcgatgcagcaagaaaggagagaggatctgattgtgaaaattagttggctcttctcttagtcttcctctttgatatttttgtgcagttttctttactgaagttggtggatccacacttgatagccatcacggttttgttgtcgagtatgggatggatagagatgttgacttgggtaaatttttgtatgcttttgagtacgggcacacttttaccctttctttaagtgaattttttaccttatcaaaaaaaagttattgtttgtttagtacttattggggtcagctattgctttgaagtgcctcaaagcctttttggctctgtgagggacattgtcttgcatctcaaccaatttaattttcaggttttcatgttgatgactcagaagtaactttaaatgtgtgcttgggtaagcaattctctggtggagagctgttcttccgtggagtgcggtgtgagaagcatgtaaatactgaaacacaacctgaggtaattattgttccgttgtttgattaactgtgcacgagaaatctctgtttcaataggaagccatgtttccattatttcatatttatcaacaaaaaaattccattatttcctatgtatttttgtttaaatggttattgtgttgtcgaaactagtagctttttgcacagtgcccttactgtcaacaacctggtaaccaagtgtattgcaactttttcagagaaaatgctgactgtttattgtgataatttgaagtcgtgataaatgttaaacctgagtttcaaagctggatccatgacaatcttcttgatcacgtgccggaacggaaaaaggcagaggactgctcttatctctttttacttttacaagtcaaaatgattccattgatatccaccatacagtgtgaatgaacgataagcttcaggtgaaaaaacggaaacctccaactatataaagaatatgacatgtcttctttacaccagaagtacaaatgaaacaaaatgtagatttaactctccacattggactctcaaccccttcaaacatttcttctgctccttctccatattagccaattaaagaggcacaactttccattattcgcttatactggcatccaactggtggtaccttttattggcaccttactttgaatgcagatttgcttgctttatttctccatagtaatcagtgatgatgaatatatgctgtgttattaccaagtttatcagctcattctcgaagtctacatatggtttaaatactgaagaaagaatgttgttagctccacgttatttgtgtgttagagtatatatcatcaaattcaaaatacaacttatgcatgtcaagagcattcactatggatttggaataatttaacaggagatctttgattactcccatgtcacggggcgtgcagtgcttcatcgtggtcgccatcggcatggtgctagagcaacaacatcggggcagaggatcaacttgttgttgtggtgcagaaggtattagatgctgttgccttgctattttgatcgtttccactagacaatttgcttcaaacacagtcgtgaaaatttgttattgttggaatatcctgttaccgctgcattacctactgtttgaagttttaagctgtgcttcataattgtttgagaacagcagtggatgcagctctttggcaacaggttcatctgaacctagtattttttccgcggtatgtgaaaacccgctaaatttcaacaaataaaaaagggcagcccagcacacaaagcatctcgcattcacacagggtccggggaagggccgcatcctaaggggtgtgatgtagacagcctacactaattccactgctcgaaccggtgacctataggtcataccgagacaactttctcgtcgctctaaggctctccttcttaaatttcaacaaatattagatctaaacccatactttttagaagaacaatgagttcagagctaagaaccttaaaggtcaaacccatctaagtttaaatccttgtctgcctctgtttaagtatgcaatattgatgcttaactacggtctccattttatctgcatagtcctccttgatgcagatatttggatgttttccattttatttctggcatcagtgcttcaagtactgaaagtagtttatgtatatcaactttcaatgatatgaggagaagtagtgtaaagtgacggtggggaaaggagcgaatactgtcttataatcatgaaaacatgatgctgatattccttgaggcacctaaatatatgtgccatgctgagttggcaactgaaaatggcatgagttaacttggaatagcatagtttagcatgtttgtagaaacgttgattaaatggttacattatatctagatctcaactttttcccttggccattgatagtggttggtcatacagacatctactagttatcgtgatttgtcaaattttttatggatacctgattacctggtggttatggtatcactcattctcctttttcacaaaataaaagaagagttttgataaacagctgaatgcatatcatgctttctggaaaagcttttctcaagaattggagatgcacatattattgattttctttttcagtgatgataggtaacttcatataggataaattcgttttgcactaactgttttacatggacagtgtgcttcatggtattcctaaaccttgaaccatgttttgctcatgtttggcttcaaacttatcaggattaaaattgctggaggtattgctaagatgctaagaaaaatctgatttatacaaggcttcacttcatatgatgcaaaatctttgcttggagtatctaattgtaactgctttttcaagaggggatggtccggtgttggtaaaagtgcataacattatacttgttccaactaaataatttgttttacttgtcaataaaaattgtatgtaaagatatgaacttctttgctgcaactcaatcagaccagatctcaataattcggatgtcttacttttattcatcttccagaatcattgaatacctgatagttgctatctttcccttacagttctgtctttagagagctaaggaagtaccagaaagacttttccggctggtgtgcagagtgccagcgcgagaagaaggaaaggcaacgactgtccattgctgctactaaattggtaagcaataattgtctcttgtaataactttaacaaatagttgacaagctctgcttatgcattatgacattaaaaggtgaaatatagttagagctggttgaagtatttttctaaattattttgtcatttgtcctttatgttttccaggagctgctgaaaagagaaggggaagctgctacatag

SEQ ID NO: 19 - protein, 397 aa, Nicotiana tabacum
MSQDGSAAATMDRKKDSQSTTNPTRNGNGNGNGGTATNGAVYPSLNSLRLRLNPSIDHKSDNYEDLQLDFSPLLFSSLERYLPPTLLNSSRDHKVHYMREILLKYCPEGERTRVQKHREYRQKIISNYQPLHRELYTMHAANFFVPSFLKAISENTEESYRNIMSEPSPGVLTFEMLQPRFCEMMLAEVENFERWVRETKFRIMRPNTMNKFGAVLDDFGLETMLDKLMEDFIRPISRVFFTEVGGSTLDSHHGFVVEYGMDRDVDLGFHVDDSEVTLNVCLGKQFSGGELFFRGVRCEKHVNTETQPEEIFDYSHVTGRAVLHRGRHRHGARATTSGQRINLLLWCRSSVFRELRKYQKDFSGWCAECQREKKERQRLSIAATKLELLKREGEAAT

SEQ ID NO: 20 - DNA, 490 bp, Artificial Sequence
  synthetically-generated oligonucleotide
aattggatccatgtctcaagatggctcagcagcagcaacaatggatcggaagaaggattctcaatcaacaacaaaccctacccgaaatggtaacggtaacggtaacggcggaacagcaacaaacggcgccgtttacccgtcactcaattctctgaggttgcgtttaaactaataagatcttcaacacctacaccatttttttaatcactactacccattgcattgaacaaacttccaagttcttcttagcttcagattaagaaagtaccctttcttggctttgttgatgtggtaccattgtccattgtcttgtgtgtttccgtttaaacgcaacctcagagaattgagtgacgggtaaacggcgccgtttgttgctgttccgccgttaccgttaccgttaccatttcgggtagggtttgttgttgattgagaatccttcttccgatccattgttgctgctgctgagccatcttgagacattctagaaatt